European Patent Application EP 4 446 414 A1, published October 16, 2024. Title: Antisense oligonucleotide complex. Applicant: Liid Pharmaceuticals, Inc. The sequence listing filed with the application follows.

SEQUENCE LISTING (69 sequences)

SEQ ID NO: 1 - DNA, 14 bp, synthetic construct
  misc_feature 1..14: note = mPCS1
  modified_base 1: mod_base = OTHER; note = 2 x GalNAcapd-linked nucleotide
  modified_base 1..3: mod_base = OTHER; note = LNA
  modified_base 12..13: mod_base = OTHER; note = LNA
  source 1..14: mol_type = other DNA
acaccaagttctcc

SEQ ID NO: 2 - DNA, 14 bp, synthetic construct
  misc_feature 1..14: note = mPCS1NoG
  modified_base 1..3: mod_base = OTHER; note = LNA
  modified_base 12..13: mod_base = OTHER; note = LNA
  source 1..14: mol_type = other DNA
acaccaagttctcc

SEQ ID NO: 3 - DNA, 12 bp, synthetic construct
  misc_feature 1..12: note = apPNA(12)-mPCS1
  modified_base 1..12: mod_base = OTHER; note = PNA
  source 1..12: mol_type = other DNA
ggagaacttggt

SEQ ID NO: 4 - DNA, 11 bp, synthetic construct
  misc_feature 1..11: note = apPNA(11)-mPCS1
  modified_base 1..11: mod_base = OTHER; note = PNA
  source 1..11: mol_type = other DNA
ggagaacttgg

SEQ ID NO: 5 - DNA, 10 bp, synthetic construct
  misc_feature 1..10: note = apPNA(10)-mPCS1
  modified_base 1..10: mod_base = OTHER; note = PNA
  source 1..10: mol_type = other DNA
ggagaacttg

SEQ ID NO: 6 - RNA, 14 nt, synthetic construct
  misc_feature 1..14: note = cRNA(14)-mPCS1
  source 1..14: mol_type = other RNA
ggagaacttggtgt

SEQ ID NO: 7 - DNA, 14 bp, synthetic construct
  misc_feature 1..14: note = mPCS1NoGaf
  modified_base 1..3: mod_base = OTHER; note = LNA
  modified_base 12..13: mod_base = OTHER; note = LNA
  modified_base 14: mod_base = OTHER; note = AlexaFluor647-linked nucleotide
  source 1..14: mol_type = other DNA
acaccaagttctcc

SEQ ID NO: 8 - DNA, 14 bp, synthetic construct
  misc_feature 1..14: note = mPCS1B
  modified_base 1: mod_base = OTHER; note = biotin-linked nucleotide
  modified_base 1..3: mod_base = OTHER; note = LNA
  modified_base 12..13: mod_base = OTHER; note = LNA
  source 1..14: mol_type = other DNA
acaccaagttctcc

SEQ ID NO: 9 - DNA, 13 bp, synthetic construct
  misc_feature 1..13: note = GN6
  modified_base 1: mod_base = OTHER; note = 3 x GalNAchp-linked nucleotide
  modified_base 1..2: mod_base = OTHER; note = LNA
  modified_base 11..13: mod_base = OTHER; note = LNA
  source 1..13: mol_type = other DNA
gcattggtattca

SEQ ID NO: 10 - DNA, 12 bp, synthetic construct
  misc_feature 1..12: note = apPNA(12)-GN6
  modified_base 1..12: mod_base = OTHER; note = PNA
  source 1..12: mol_type = other DNA
tgaataccaatg

SEQ ID NO: 11 - DNA, 11 bp, synthetic construct
  misc_feature 1..11: note = apPNA(11)-GN6
  modified_base 1..11: mod_base = OTHER; note = PNA
  source 1..11: mol_type = other DNA
tgaataccaat

SEQ ID NO: 12 - DNA, 10 bp, synthetic construct
  misc_feature 1..10: note = apPNA(10)-GN6
  modified_base 1..10: mod_base = OTHER; note = PNA
  source 1..10: mol_type = other DNA
tgaataccaa

SEQ ID NO: 13 - DNA, 10 bp, synthetic construct
  misc_feature 1..10: note = apPNA(C10)-GN6
  source 1..10: mol_type = other DNA
ataccaatgc

SEQ ID NO: 14 - RNA, 13 nt, synthetic construct
  misc_feature 1..13: note = cRNA-GN6
  source 1..13: mol_type = other RNA
tgaataccaatgc

SEQ ID NO: 15 - DNA, 13 bp, synthetic construct
  misc_feature 1..13: note = hApo1
  modified_base 1: mod_base = OTHER; note = 2 x GalNAcapd-linked nucleotide
  modified_base 1..2: mod_base = OTHER; note = LNA
  modified_base 11..13: mod_base = OTHER; note = LNA
  source 1..13: mol_type = other DNA
aatggccagcttg

SEQ ID NO: 16 - DNA, 10 bp, synthetic construct
  misc_feature 1..10: note = apPNA(C10)-hApo1
  modified_base 1..10: mod_base = OTHER; note = PNA
  source 1..10: mol_type = other DNA
gctggccatt

SEQ ID NO: 17 - DNA, 11 bp, synthetic construct
  misc_feature 1..11: note = apPNA(C11)-hApo1
  modified_base 1..11: mod_base = OTHER; note = PNA
  source 1..11: mol_type = other DNA
agctggccatt

SEQ ID NO: 18 - DNA, 12 bp, synthetic construct
  misc_feature 1..12: note = apPNA(C12)-hApo1
  modified_base 1..12: mod_base = OTHER; note = PNA
  source 1..12: mol_type = other DNA
aagctggccatt

SEQ ID NO: 19 - DNA, 13 bp, synthetic construct
  misc_feature 1..13: note = apPNA(C13)-hApo1
  modified_base 1..13: mod_base = OTHER; note = PNA
  source 1..13: mol_type = other DNA
caagctggccatt

SEQ ID NO: 20 - RNA, 13 nt, synthetic construct
  misc_feature 1..13: note = cRNA-hApo1
  source 1..13: mol_type = other RNA
caagctggccatt

SEQ ID NO: 21 - DNA, 20 bp, synthetic construct
  misc_feature 1..20: note = PCR Primer(mPCSK9-F)
  source 1..20: mol_type = other DNA
tcagttctgcacacctccag

SEQ ID NO: 22 - DNA, 20 bp, synthetic construct
  misc_feature 1..20: note = PCR Primer(mPCSK9-R)
  source 1..20: mol_type = other DNA
gggtaaggtgcggtaagtcc

SEQ ID NO: 23 - DNA, 20 bp, synthetic construct
  misc_feature 1..20: note = PCR Primer(mGAPDH-F)
  source 1..20: mol_type = other DNA
tgtgtccgtcgtggatctga

SEQ ID NO: 24 - DNA, 21 bp, synthetic construct
  misc_feature 1..21: note = PCR Primer(mGAPDH-R)
  source 1..21: mol_type = other DNA
ttgctgttgaagtcgcaggag

SEQ ID NO: 25 - DNA, 24 bp, synthetic construct
  misc_feature 1..24: note = PCR Primer(mApoB-F)
  source 1..24: mol_type = other DNA
tcctcggtgagttcaatgactttc

SEQ ID NO: 26 - DNA, 23 bp, synthetic construct
  misc_feature 1..23: note = PCR Primer(mApoB-R)
  source 1..23: mol_type = other DNA
tggacctgctgtagcttgtagga

SEQ ID NO: 27 - DNA, 20 bp, synthetic construct
  misc_feature 1..20: note = PCR Primer(Plastin1-Fw)
  source 1..20: mol_type = other DNA
gtgaagccgaagatggtgat

SEQ ID NO: 28 - DNA, 20 bp, synthetic construct
  misc_feature 1..20: note = PCR Primer(Plastin1-Rv)
  source 1..20: mol_type = other DNA
gtttggtgcgtacagtgtgg

SEQ ID NO: 29 - DNA, 20 bp, synthetic construct
  misc_feature 1..20: note = PCR Primer(Lrp2-Fw)
  source 1..20: mol_type = other DNA
ggttcgttatggcagtcgtt

SEQ ID NO: 30 - DNA, 20 bp, synthetic construct
  misc_feature 1..20: note = PCR Primer(Lrp2-Rv)
  source 1..20: mol_type = other DNA
tgctggcttggaagactttt

SEQ ID NO: 31 - DNA, 20 bp, synthetic construct
  misc_feature 1..20: note = PCR Primer(Atp5c1-Fw)
  source 1..20: mol_type = other DNA
tgaagccctgtgaaacactg

SEQ ID NO: 32 - DNA, 20 bp, synthetic construct
  misc_feature 1..20: note = PCR Primer(Atp5c1-Rv)
  source 1..20: mol_type = other DNA
agcaaagagtcggatggcta

SEQ ID NO: 33 - DNA, 20 bp, synthetic construct
  misc_feature 1..20: note = PCR Primer(Pirin-Fw)
  source 1..20: mol_type = other DNA
catttcaggagaagccttgg

SEQ ID NO: 34 - DNA, 20 bp, synthetic construct
  misc_feature 1..20: note = PCR Primer(Pirin-Rv)
  source 1..20: mol_type = other DNA
aggaataggctgggaatgct

SEQ ID NO: 35 - DNA, 20 bp, synthetic construct
  misc_feature 1..20: note = PCR Primer(Dpyd-Fw)
  source 1..20: mol_type = other DNA
ctcgcaaaagcctattcctg

SEQ ID NO: 36 - DNA, 20 bp, synthetic construct
  misc_feature 1..20: note = PCR Primer(Dpyd-Rv)
  source 1..20: mol_type = other DNA
atcagggccacaacttgttc

SEQ ID NO: 37 - DNA, 12 bp, synthetic construct
  misc_feature 1..12: note = antisense strand of double-stranded nucleic acid (1)
  modified_base 1..2: mod_base = OTHER; note = LNA
  modified_base 11..12: mod_base = OTHER; note = LNA
  source 1..12: mol_type = other DNA
gcattggtattc

SEQ ID NO: 38 - DNA, 10 bp, synthetic construct
  misc_feature 1..10: note = complementary strand of double-stranded nucleic acid (1)
  modified_base 1..10: mod_base = OTHER; note = PNA
  source 1..10: mol_type = other DNA
  modified_base 4: mod_base = OTHER; note = deoxyuridine
  modified_base 10: mod_base = OTHER; note = deoxyuridine
gaataccaat

SEQ ID NO: 39 - DNA, 10 bp, synthetic construct
  misc_feature 1..10: note = complementary strand of double-stranded nucleic acid (2)
  modified_base 1..10: mod_base = OTHER; note = PNA
  source 1..10: mol_type = other DNA
gaataccaat

SEQ ID NO: 40 - RNA, 14 nt, synthetic construct
  source 1..14: mol_type = other RNA
  misc_feature 2..14: note = phosphorothioate phosphate
  modified_base 1..2: mod_base = gm
  modified_base 3: mod_base = OTHER; note = 2'-O-methyladenosine
  modified_base 12: mod_base = um
  modified_base 13: mod_base = gm
  modified_base 14: mod_base = um
ggagaacttggtgt

SEQ ID NO: 41 - DNA, 13 bp, synthetic construct
  source 1..13: mol_type = other DNA
  modified_base 1..2: mod_base = OTHER; note = LNA
  modified_base 11..13: mod_base = OTHER; note = LNA
  modified_base 1: mod_base = OTHER; note = TAMRA-linked nucleotide
aatggccagcttg

SEQ ID NO: 42 - RNA, 13 nt, Homo sapiens
  source 1..13: mol_type = mRNA
  modified_base 13: mod_base = OTHER; note = BHQ2-linked nucleotide
caagctggccatt

SEQ ID NO: 43 - RNA, 13 nt, Homo sapiens
  source 1..13: mol_type = mRNA
  modified_base 13: mod_base = OTHER; note = BHQ2-linked nucleotide
caagcgggccatt

SEQ ID NO: 44 - RNA, 13 nt, Homo sapiens
  source 1..13: mol_type = mRNA
  modified_base 13: mod_base = OTHER; note = BHQ2-linked nucleotide
caaggtggccatt

SEQ ID NO: 45 - RNA, 13 nt, Homo sapiens
  source 1..13: mol_type = mRNA
  modified_base 13: mod_base = OTHER; note = BHQ2-linked nucleotide
caagttggccatt

SEQ ID NO: 46 - DNA, 18 bp, synthetic construct
  source 1..18: mol_type = other DNA
  modified_base 1..3: mod_base = OTHER; note = LNA
  modified_base 16..17: mod_base = OTHER; note = LNA
  modified_base 1: mod_base = OTHER; note = 3 x GalNAcapd-linked nucleotide
ctccatgacacagcatta

SEQ ID NO: 47 - DNA, 18 bp, synthetic construct
  source 1..18: mol_type = other DNA
  modified_base 1..3: mod_base = OTHER; note = LNA
  modified_base 16..17: mod_base = OTHER; note = LNA
ctccatgacacagcatta

SEQ ID NO: 48 - DNA, 18 bp, synthetic construct
  source 1..18: mol_type = other DNA
  modified_base 1..3: mod_base = OTHER; note = LNA
  modified_base 16..17: mod_base = OTHER; note = LNA
  modified_base 1: mod_base = OTHER; note = biotin-linked nucleotide
ctccatgacacagcatta

SEQ ID NO: 49 - DNA, 14 bp, synthetic construct
  source 1..14: mol_type = other DNA
  modified_base 1..14: mod_base = OTHER; note = parallel PNA
tactgtgtcgtaat

SEQ ID NO: 50 - DNA, 15 bp, synthetic construct
  source 1..15: mol_type = other DNA
  modified_base 1..15: mod_base = OTHER; note = parallel PNA
gtactgtgtcgtaat

SEQ ID NO: 51 - DNA, 16 bp, synthetic construct
  source 1..16: mol_type = other DNA
  modified_base 1..16: mod_base = OTHER; note = parallel PNA
ggtactgtgtcgtaat

SEQ ID NO: 52 - DNA, 17 bp, synthetic construct
  source 1..17: mol_type = other DNA
  modified_base 1..17: mod_base = OTHER; note = parallel PNA
aggtactgtgtcgtaat

SEQ ID NO: 53 - DNA, 18 bp, synthetic construct
  source 1..18: mol_type = other DNA
  modified_base 1..18: mod_base = OTHER; note = parallel PNA
gaggtactgtgtcgtaat

SEQ ID NO: 54 - RNA, 18 nt, synthetic construct
  source 1..18: mol_type = other RNA
taatgctgtgtcatggag

SEQ ID NO: 55 - DNA, 14 bp, synthetic construct
  source 1..14: mol_type = other DNA
  modified_base 1..3: mod_base = OTHER; note = LNA
  modified_base 12..13: mod_base = OTHER; note = LNA
  modified_base 1: mod_base = OTHER; note = 4 x GalNAcapd-linked nucleotide
agaatactgtccct

SEQ ID NO: 56 - DNA, 10 bp, synthetic construct
  source 1..10: mol_type = other DNA
  misc_feature 1..10: note = 3-0PNA(10)
  modified_base 1..10: mod_base = OTHER; note = PNA
agggacagta

SEQ ID NO: 57 - DNA, 14 bp, synthetic construct
  source 1..14: mol_type = other DNA
  modified_base 1..2: mod_base = OTHER; note = LNA
  modified_base 12..13: mod_base = OTHER; note = LNA
  modified_base 1: mod_base = OTHER; note = 3 x GalNAchp-linked nucleotide
cctaggagttcgca

SEQ ID NO: 58 - DNA, 24 bp, synthetic construct
  source 1..24: mol_type = other DNA
  misc_feature 1..24: note = PCR Primer(hApoB-F)
ttctcaagagttacagcagatcca

SEQ ID NO: 59 - DNA, 25 bp, synthetic construct
  source 1..25: mol_type = other DNA
  misc_feature 1..25: note = PCR Primer(hApoB-R)
tggaagtccttaagagcaactaaca

SEQ ID NO: 60 - DNA, 20 bp, synthetic construct
  source 1..20: mol_type = other DNA
  misc_feature 1..20: note = PCR Primer(hCopg-F)
ccatgcattgggagtcctgt

SEQ ID NO: 61 - DNA, 20 bp, synthetic construct
  source 1..20: mol_type = other DNA
  misc_feature 1..20: note = PCR Primer(hCopg-R)
actggcaattcggatcagca

SEQ ID NO: 62 - DNA, 20 bp, synthetic construct
  source 1..20: mol_type = other DNA
  misc_feature 1..20: note = PCR Primer(hMast2-F)
tgactttcgctgagaacccc

SEQ ID NO: 63 - DNA, 20 bp, synthetic construct
  source 1..20: mol_type = other DNA
  misc_feature 1..20: note = PCR Primer(hMast2-R)
tcttcagcagagtggcacag

SEQ ID NO: 64 - DNA, 20 bp, synthetic construct
  source 1..20: mol_type = other DNA
  misc_feature 1..20: note = PCR Primer(hHltf-F)
cctgtgccgttttcttgctc

SEQ ID NO: 65 - DNA, 20 bp, synthetic construct
  source 1..20: mol_type = other DNA
  misc_feature 1..20: note = PCR Primer(hHltf-R)
ccctgcagaaaggtcttggt

SEQ ID NO: 66 - DNA, 20 bp, synthetic construct
  source 1..20: mol_type = other DNA
  misc_feature 1..20: note = PCR Primer(hGapdh-F)
gcaccgtcaaggctgagaac

SEQ ID NO: 67 - DNA, 19 bp, synthetic construct
  source 1..19: mol_type = other DNA
  misc_feature 1..19: note = PCR Primer(hGapdh-R)
tggtgaagacgccagtgga

SEQ ID NO: 68 - DNA, 20 bp, synthetic construct
  source 1..20: mol_type = other DNA
  misc_feature 1..20: note = PCR Primer(mAcsl1-F)
aggtgcttcagcccaccatc

SEQ ID NO: 69 - DNA, 22 bp, synthetic construct
  source 1..22: mol_type = other DNA
  misc_feature 1..22: note = PCR Primer(mAcsl1-R)
aaagtccaacagccatcgcttc